European Patent Application EP 4 759 932 A1, published June 17, 2026. Title: 基于mRNA-LNP的诱导多能性干细胞的重编程方法. Applicant: 宜明（苏州）细胞生物科技有限公司. The sequence listing filed with the application follows.

SEQUENCE LISTING (14 sequences)

SEQ ID NO: 1 - protein, 360 aa, Homo sapiens
MAGHLASDFAFSPPPGGGGDGPGGPEPGWVDPRTWLSFQGPPGGPGIGPGVGPGSEVWGIPPCPPPYEFCGGMAYCGPQVGVGLVPQGGLETSQPEGEAGVGVESNSDGASPEPCTVTPGAVKLEKEKLEQNPEESQDIKALQKELEQFAKLLKQKRITLGYTQADVGLTLGVLFGKVFSQTTICRFEALQLSFKNMCKLRPLLQKWVEEADNNENLQEICKAETLVQARKRKRTSIENRVRGNLENLFLQCPKPTLQQISHIAQQLGLEKDVVRVWFCNRRQKGKRSSSDYAQREDFEAAGSPFSGGPVSFPLAPGPHFGTPGYGSPHFTALYSSVPFPEGEAFPPVSVTTLGSPMHSN

SEQ ID NO: 2 - protein, 470 aa, Homo sapiens
MAVSDALLPSFSTFASGPAGREKTLRQAGAPNNRWREELSHMKRLPPVLPGRPYDLAAATVATDLESGGAGAACGGSNLAPLPRRETEEFNDLLDLDFILSNSLTHPPESVAATVSSSASASSSSSPSSSGPASAPSTCSFTYPIRAGNDPGVAPGGTGGGLLYGRESAPPPTAPFNLADINDVSPSGGFVAELLRPELDPVYIPPQQPQPPGGGLMGKFVLKASLSAPGSEYGSPSVISVSKGSPDGSHPVVVAPYNGGPPRTCPKIKQEAVSSCTHLGAGPPLSNGHRPAAHDFPLGRQLPSRTTPTLGLEEVLSSRDCHPALPLPPGFHPHPGPNYPSFLPDQMQPQVPPLHYQELMPPGSCMPEEPKPKRGRRSWPRKRTATHTCDYAGCGKTYTKSSHLKAHLRTHTGEKPYHCDWDGCGWKFARSDELTRHYRKHTGHRPFQCQKCDRAFSRSDHLALHMKRHF

SEQ ID NO: 3 - protein, 317 aa, Homo sapiens
MYNMMETELKPPGPQQTSGGGGGNSTAAAAGGNQKNSPDRVKRPMNAFMVWSRGQRRKMAQENPKMHNSEISKRLGAEWKLLSETEKRPFIDEAKRLRALHMKEHPDYKYRPRRKTKTLMKKDKYTLPGGLLAPGGNSMASGVGVGAGLGAGVNQRMDSYAHMNGWSNGSYSMMQDQLGYPQHPGLNAHGAAQMQPMHRYDVSALQYNSMTSSQTYMNGSPTYSMSYSQQGTPGMALGSMGSVVKSEASSSPPVVTSSSHSRAPCQAGDLRDMISMYLPGAEVPEPAAPSRLHMSQHYQSGPVPGTAINGTLPLSHM

SEQ ID NO: 4 - protein, 440 aa, Homo sapiens
MGPLNVSFTNRNYDLDYDSVQPYFYCDEEENFYQQQQQSELQPPAPSEDIWKKFELLPTPPLSPSRRSGLCSPSYVAVTPFSLRGDNDGGGGSFSTADQLEMVTELLGGDMVNQSFICDPDDETFIKNIIIQDCMWSGFSAAAKLVSEKLASYQAARKDSGSPNPARGHSVCSTSSLYLQDLSAAASECIDPSVVFPYPLNDSSSPKSCASQDSSAFSPSSDSLLSSTESSPQGSPEPLVLHEETPPTTSSDSEEEQEDEEEIDVVSVEKRQAPGKRSESGSPSAGGHSKPPHSPLVLKRCHVSTHQHNYAAPPSTRKDYPAAKRVKLDSVRVLRQISNNRKCTSPRSSDTEENVKRRTHNVLERQRRNELKRSFFALRDQIPELENNEKAPKVVILKKATAYILSVQAEEQKLISEEDLLRKRREQLKHKLEQLRNSCA

SEQ ID NO: 5 - protein, 209 aa, Homo sapiens
MGSVSNQQFAGGCAKAAEEAPEEAPEDAARAADEPQLLHGAGICKWFNVRMGFGFLSMTARAGVALDPPVDVFVHQSKLHMEGFRSLKEGEAVEFTFKKSAKGLESIRVTGPGGVFCIGSERRPKGKSMQKRRSKGDRCYNCGGLDHHAKECKLPPQPKKCHFCQSISHMVASCPLKAQQGPSAQGKPTYFREEEEEIHSPTLLPEAQN

SEQ ID NO: 6 - protein, 620 aa, Homo sapiens
MAEARTSLSAHCRGPLATGLHPDLDLPGRSLATPAPSCYLLGSEPSSGLGLQPETHLPEGSLKRCCVLGLPPTSPASSSPCASSDVTSIIRSSQTSLVTCVNGLRSPPLTGDLGGPSKRARPGPASTDSHEGSLQLEACRKASFLKQEPADEFSELFGPHQQGLPPPYPLSQLPPGPSLGGLGLGLAGRVVAGRQACRWVDCCAAYEQQEELVRHIEKSHIDQRKGEDFTCFWAGCVRRYKPFNARYKLLIHMRVHSGEKPNKCMFEGCSKAFSRLENLKIHLRSHTGEKPYLCQHPGCQKAFSNSSDRAKHQRTHLDTKPYACQIPGCSKRYTDPSSLRKHVKAHSAKEQQVRKKLHAGPDTEADVLTECLVLQQLHTSTQLAASDGKGGCGLGQELLPGVYPGSITPHNGLASGLLPPAHDVPSRHHPLDATTSSHHHLSPLPMAESTRDGLGPGLLSPIVSPLKGLGPPPLPPSSQSHSPGGQPFPTLPSKPSYPPFQSPPPPPLPSPQGYQGSFHSIQSCFPYGDCYRMAEPAAGGDGLVGETHGFNPLRPNGYHSLSTPLPATGYEALAEASCPTALPQQPSEDVVSSGPEDCGFFPNGAFDHCLGHIPSIYTDT

SEQ ID NO: 7 - RNA, 1579 nt, synthetic construct
  source 1..1579: mol_type = other RNA
ggaaaaaaggaaagtgcacttggaagagatccaagtgggcaacttgaagaacaagtgccaaatagcacttctgtcatgctggatgtcagggctctttgtccactttgtatagccgctggcttatagaaggtgctcgataaatctcttgaatttaaaaatcaattaggatgcctctatagtgaaaaagatacagtaaagatgagggataatcaatttaaaaaatgagtaagtacacacaaagcactttatccattcttatgacacctgttacttttttgctgtgtttgtgtgtatgcatgccatgttatagtttgtgggaccctcaaagcaagctggggagagtatatactgaatttagcttctgagacatgatgctcttcctttttaattaacccagaacttagcagcttatctatttctctaatctcaaaacatccttaaactgggggtgatacttgagtgagagaattttgcaggtattaaatgaactatcttcttttttttttttctttgagacagagtcttgctctgtcacccaggctggagtgcagtggcgtgatctcagctcactgcaacctccgcctcccgggttcaagtgattctcctgcctcagcctcctgagtagctgggattacagtcccaggacatcaaagctctgcagaaagaactcgagcaatttgccaagctcctgaagcagaagaggatcaccctgggatatacacaggccgatgtggggctcaccctgggggttctatttgggaaggtattcagccaaacgaccatctgccgctttgaggctctgcagcttagcttcaagaacatgtgtaagctgcggcccttgctgcagaagtgggtggaggaagctgacaacaatgaaaatcttcaggagatatgcaaagcagaaaccctcgtgcaggcccgaaagagaaagcgaaccagtatcgagaaccgagtgagaggcaacctggagaatttgttcctgcagtgcccgaaacccacactgcagcagatcagccacatcgcccagcagcttgggctcgagaaggatgtggtccgagtgtggttctgtaaccggcgccagaagggcaagcgatcaagcagcgactatgcacaacgagaggattttgaggctgctgggtctcctttctcagggggaccagtgtcctttcctctggccccagggccccattttggtaccccaggctatgggagccctcacttcactgcactgtactcctcggtccctttccctgagggggaagcctttccccctgtctccgtcaccactctgggctctcccatgcattcaaactgaggtgcctgcccttctaggaatgggggacagggggaggggaggagctagggaaagaaaacctggagtttgtgccagggtttttgggattaagttcttcattcactaaggaaggaattgggaacacaaagggtgggggcaggggagtttggggcaactggttggagggaaggtgaagttcaatgatgctcttgattttaatcccacatcatgtatcacttttttcttaaataaagaagcctgggacacagtagatagacacactta

SEQ ID NO: 8 - RNA, 2936 nt, synthetic construct
  source 1..2936: mol_type = other RNA
ggcagtttcccgaccagagagaacgaacgtgtctgcgggcgcgcggggagcagaggcggtggcgggcggcggcggcaccgggagccgccgagtgaccctcccccgcccctctggccccccaccctcccacccgcccgtggcccgcgcccatggccgcgcgcgctccacacaactcaccggagtccgcgccttgcgccgccgaccagttcgcagctccgcgccacggcagccagtctcacctggcggcaccgcccgcccaccgccccggccacagcccctgcgcccacggcagcactcgaggcgaccgcgacagtggtgggggacgctgctgagtggaagagagcgcagcccggccaccggacctacttactcgccttgctgattgtctatttttgcgtttacaacttttctaagaacttttgtatacaaaggaactttttaaaaaagacgcttccaagttatatttaatccaaagaagaaggatctcggccaatttggggttttgggttttggcttcgtttcttctcttcgttgactttggggttcaggtgccccagctgcttcgggctgccgaggaccttctgggcccccacattaatgaggcagccacctggcgagtctgacatggctgtcagcgacgcgctgctcccatctttctccacgttcgcgtctggcccggcgggaagggagaagacactgcgtcaagcaggtgccccgaataaccgctggcgggaggagctctcccacatgaagcgacttcccccagtgcttcccggccgcccctatgacctggcggcggcgaccgtggccacagacctggagagcggcggagccggtgcggcttgcggcggtagcaacctggcgcccctacctcggagagagaccgaggagttcaacgatctcctggacctggactttattctctccaattcgctgacccatcctccggagtcagtggccgccaccgtgtcctcgtcagcgtcagcctcctcttcgtcgtcgccgtcgagcagcggccctgccagcgcgccctccacctgcagcttcacctatccgatccgggccgggaacgacccgggcgtggcgccgggcggcacgggcggaggcctcctctatggcagggagtccgctccccctccgacggctcccttcaacctggcggacatcaacgacgtgagcccctcgggcggcttcgtggccgagctcctgcggccagaattggacccggtgtacattccgccgcagcagccgcagccgccaggtggcgggctgatgggcaagttcgtgctgaaggcgtcgctgagcgcccctggcagcgagtacggcagcccgtcggtcatcagcgtcagcaaaggcagccctgacggcagccacccggtggtggtggcgccctacaacggcgggccgccgcgcacgtgccccaagatcaagcaggaggcggtctcttcgtgcacccacttgggcgctggaccccctctcagcaatggccaccggccggctgcacacgacttccccctggggcggcagctccccagcaggactaccccgaccctgggtcttgaggaagtgctgagcagcagggactgtcaccctgccctgccgcttcctcccggcttccatccccacccggggcccaattacccatccttcctgcccgatcagatgcagccgcaagtcccgccgctccattaccaagagctcatgccacccggttcctgcatgccagaggagcccaagccaaagaggggaagacgatcgtggccccggaaaaggaccgccacccacacttgtgattacgcgggctgcggcaaaacctacacaaagagttcccatctcaaggcacacctgcgaacccacacaggtgagaaaccttaccactgtgactgggacggctgtggatggaaattcgcccgctcagatgaactgaccaggcactaccgtaaacacacggggcaccgcccgttccagtgccaaaaatgcgaccgagcattttccaggtcggaccacctcgccttacacatgaagaggcatttttaaatcccagacagtggatatgacccacactgccagaagagaattcagtattttttacttttcacactgtcttcccgatgagggaaggagcccagccagaaagcactacaatcatggtcaagttcccaactgagtcatcttgtgagtggataatcaggaaaaatgaggaatccaaaagacaaaaatcaaagaacagatggggtctgtgactggatcttctatcattccaattctaaatccgacttgaatattcctggacttacaaaatgccaagggggtgactggaagttgtggatatcagggtataaattatatccgtgagttgggggagggaagaccagaattcccttgaattgtgtattgatgcaatataagcataaaagatcaccttgtattctctttaccttctaaaagccattattatgatgttagaagaagaggaagaaattcaggtacagaaaacatgtttaaatagcctaaatgatggtgcttggtgagtcttggttctaaaggtaccaaacaaggaagccaaagttttcaaactgctgcatactttgacaaggaaaatctatatttgtcttccgatcaacatttatgacctaagtcaggtaatatacctggtttacttctttagcatttttatgcagacagtctgttatgcactgtggtttcagatgtgcaataatttgtacaatggtttattcccaagtatgccttaagcagaacaaatgtgtttttctatatagttccttgccttaataaatatgtaatataaatttaagcaaacgtctattttgtatatttgtaaactacaaagtaaaatgaacattttgtggagtttgtattttgcatactcaaggtgagaattaagttttaaataaacctataatattttatctgaa

SEQ ID NO: 9 - RNA, 2512 nt, synthetic construct
  source 1..2512: mol_type = other RNA
gatggttgtctattaacttgttcaaaaaagtatcaggagttgtcaaggcagagaagagagtgtttgcaaaagggggaaagtagtttgctgcctctttaagactaggactgagagaaagaagaggagagagaaagaaagggagagaagtttgagccccaggcttaagcctttccaaaaaataataataacaatcatcggcggcggcaggatcggccagaggaggagggaagcgctttttttgatcctgattccagtttgcctctctctttttttcccccaaattattcttcgcctgattttcctcgcggagccctgcgctcccgacacccccgcccgcctcccctcctcctctccccccgcccgcgggccccccaaagtcccggccgggccgagggtcggcggccgccggcgggccgggcccgcgcacagcgcccgcatgtacaacatgatggagacggagctgaagccgccgggcccgcagcaaacttcggggggcggcggcggcaactccaccgcggcggcggccggcggcaaccagaaaaacagcccggaccgcgtcaagcggcccatgaatgccttcatggtgtggtcccgcgggcagcggcgcaagatggcccaggagaaccccaagatgcacaactcggagatcagcaagcgcctgggcgccgagtggaaacttttgtcggagacggagaagcggccgttcatcgacgaggctaagcggctgcgagcgctgcacatgaaggagcacccggattataaataccggccccggcggaaaaccaagacgctcatgaagaaggataagtacacgctgcccggcgggctgctggcccccggcggcaatagcatggcgagcggggtcggggtgggcgccggcctgggcgcgggcgtgaaccagcgcatggacagttacgcgcacatgaacggctggagcaacggcagctacagcatgatgcaggaccagctgggctacccgcagcacccgggcctcaatgcgcacggcgcagcgcagatgcagcccatgcaccgctacgacgtgagcgccctgcagtacaactccatgaccagctcgcagacctacatgaacggctcgcccacctacagcatgtcctactcgcagcagggcacccctggcatggctcttggctccatgggttcggtggtcaagtccgaggccagctccagcccccctgtggttacctcttcctcccactccagggcgccctgccaggccggggacctccgggacatgatcagcatgtatctccccggcgccgaggtgccggaacccgccgcccccagcagacttcacatgtcccagcactaccagagcggcccggtgcccggcacggccattaacggcacactgcccctctcacacatgtgagggccggacagcgaactggaggggggagaaattttcaaagaaaaacgagggaaatgggaggggtgcaaaagaggagagtaagaaacagcatggagaaaacccggtacgctcaaaaagaaaaaggaaaaaaaaaaatcccatcacccacagcaaatgacagctgcaaaagagaacaccaatcccatccacactcacgcaaaaaccgcgatgccgacaagaaaacttttatgagagagatcctggacttctttttgggggactatttttgtacagagaaaacctggggagggtggggagggcgggggaatggaccttgtatagatctggaggaaagaaagctacgaaaaactttttaaaagttctagtggtacggtaggagctttgcaggaagtttgcaaaagtctttaccaataatatttagagctagtctccaagcgacgaaaaaaatgttttaatatttgcaagcaacttttgtacagtatttatcgagataaacatggcaatcaaaatgtccattgtttataagctgagaatttgccaatatttttcaaggagaggcttcttgctgaattttgattctgcagctgaaatttaggacagttgcaaacgtgaaaagaagaaaattattcaaatttggacattttaattgtttaaaaattgtacaaaaggaaaaaattagaataagtactggcgaaccatctctgtggtcttgtttaaaaagggcaaaagttttagactgtactaaattttataacttactgttaaaagcaaaaatggccatgcaggttgacaccgttggtaatttataatagcttttgttcgatcccaactttccattttgttcagataaaaaaaaccatgaaattactgtgtttgaaatattttcttatggtttgtaatatttctgtaaatttattgtgatattttaaggttttcccccctttattttccgtagttgtattttaaaagattcggctctgtattatttgaatcagtctgccgagaatccatgtatatatttgaactaatatcatccttataacaggtacattttcaacttaagtttttactccattatgcacagtttgagataaataaatttttgaaatatggacactgaaa

SEQ ID NO: 10 - RNA, 4515 nt, synthetic construct
  source 1..4515: mol_type = other RNA
ggagtttattcataacgcgctctccaagtatacgtggcaatgcgttgctgggttattttaatcattctaggcatcgttttcctccttatgcctctatcattcctccctatctacactaacatcccacgctctgaacgcgcgcccattaatacccttctttcctccactctccctgggactcttgatcaaagcgcggccctttccccagccttagcgaggcgccctgcagcctggtacgcgcgtggcgtggcggtgggcgcgcagtgcgttctcggtgtggagggcagctgttccgcctgcgatgatttatactcacaggacaaggatgcggtttgtcaaacagtactgctacggaggagcagcagagaaagggagagggtttgagagggagcaaaagaaaatggtaggcgcgcgtagttaattcatgcggctctcttactctgtttacatcctagagctagagtgctcggctgcccggctgagtctcctccccaccttccccaccctccccaccctccccataagcgcccctcccgggttcccaaagcagagggcgtgggggaaaagaaaaaagatcctctctcgctaatctccgcccaccggccctttataatgcgagggtctggacggctgaggacccccgagctgtgctgctcgcggccgccaccgccgggccccggccgtccctggctcccctcctgcctcgagaagggcagggcttctcagaggcttggcgggaaaaagaacggagggagggatcgcgctgagtataaaagccggttttcggggctttatctaactcgctgtagtaattccagcgagaggcagagggagcgagcgggcggccggctagggtggaagagccgggcgagcagagctgcgctgcgggcgtcctgggaagggagatccggagcgaatagggggcttcgcctctggcccagccctcccgctgatcccccagccagcggtccgcaacccttgccgcatccacgaaactttgcccatagcagcgggcgggcactttgcactggaacttacaacacccgagcaaggacgcgactctcccgacgcggggaggctattctgcccatttggggacacttccccgccgctgccaggacccgcttctctgaaaggctctccttgcagctgcttagacgctggatttttttcgggtagtggaaaaccagcctcccgcgacgatgcccctcaacgttagcttcaccaacaggaactatgacctcgactacgactcggtgcagccgtatttctactgcgacgaggaggagaacttctaccagcagcagcagcagagcgagctgcagcccccggcgcccagcgaggatatctggaagaaattcgagctgctgcccaccccgcccctgtcccctagccgccgctccgggctctgctcgccctcctacgttgcggtcacacccttctcccttcggggagacaacgacggcggtggcgggagcttctccacggccgaccagctggagatggtgaccgagctgctgggaggagacatggtgaaccagagtttcatctgcgacccggacgacgagaccttcatcaaaaacatcatcatccaggactgtatgtggagcggcttctcggccgccgccaagctcgtctcagagaagctggcctcctaccaggctgcgcgcaaagacagcggcagcccgaaccccgcccgcggccacagcgtctgctccacctccagcttgtacctgcaggatctgagcgccgccgcctcagagtgcatcgacccctcggtggtcttcccctaccctctcaacgacagcagctcgcccaagtcctgcgcctcgcaagactccagcgccttctctccgtcctcggattctctgctctcctcgacggagtcctccccgcagggcagccccgagcccctggtgctccatgaggagacaccgcccaccaccagcagcgactctgaggaggaacaagaagatgaggaagaaatcgatgttgtttctgtggaaaagaggcaggctcctggcaaaaggtcagagtctggatcaccttctgctggaggccacagcaaacctcctcacagcccactggtcctcaagaggtgccacgtctccacacatcagcacaactacgcagcgcctccctccactcggaaggactatcctgctgccaagagggtcaagttggacagtgtcagagtcctgagacagatcagcaacaaccgaaaatgcaccagccccaggtcctcggacaccgaggagaatgtcaagaggcgaacacacaacgtcttggagcgccagaggaggaacgagctaaaacggagcttttttgccctgcgtgaccagatcccggagttggaaaacaatgaaaaggcccccaaggtagttatccttaaaaaagccacagcatacatcctgtccgtccaagcagaggagcaaaagctcatttctgaagaggacttgttgcggaaacgacgagaacagttgaaacacaaacttgaacagctacggaactcttgtgcgtaaggaaaagtaaggaaaacgattccttctaacagaaatgtcctgagcaatcacctatgaacttgtttcaaatgcatgatcaaatgcaacctcacaaccttggctgagtcttgagactgaaagatttagccataatgtaaactgcctcaaattggactttgggcataaaagaacttttttatgcttaccatcttttttttttctttaacagatttgtatttaagaattgtttttaaaaaattttaagatttacacaatgtttctctgtaaatattgccattaaatgtaaataactttaataaaacgtttatagcagttacacagaatttcaatcctagtatatagtacctagtattataggtactataaaccctaattttttttatttaagtacattttgctttttaaagttgatttttttctattgtttttagaaaaaataaaataactggcaaatatatcattgagccaaatcttaagttgtgaatgttttgtttcgtttcttccccctcccaaccaccaccatccctgtttgttttcatcaattgccccttcagagggtggtcttaagaaaggcaagagttttcctctgttgaaatgggtctgggggccttaaggtctttaagttcttggaggttctaagatgcttcctggagactatgataacagccagagttgacagttagaaggaatggcagaaggcaggtgagaaggtgagaggtaggcaaaggagatacaagaggtcaaaggtagcagttaagtacacaaagaggcataaggactggggagttgggaggaaggtgaggaagaaactcctgttactttagttaaccagtgccagtcccctgctcactccaaacccaggaattctgcccagttgatggggacacggtgggaaccagcttctgctgccttcacaaccaggcgccagtcctgtccatgggttatctcgcaaaccccagaggatctctgggaggaatgctactattaaccctatttcacaaacaaggaaatagaagagctcaaagaggttatgtaacttatctgtagccacgcagataatacaaagcagcaatctggacccattctgttcaaaacacttaacccttcgctatcatgccttggttcatctgggtctaatgtgctgagatcaagaaggtttaggacctaatggacagactcaagtcataacaatgctaagctctatttgtgtcccaagcactcctaagcattttatccctaactctacatcaaccccatgaaggagatactgttgatttccccatattagaagtagagagggaagctgaggcacacaaagactcatccacatgcccaagattcactgatagggaaaagtggaagcgagatttgaacccaggctgtttactcctaacctgtccaagccacctctcagacgacggtaggaatcagctggctgcttgtgagtacaggagttacagtccagtgggttatgttttttaagtctcaacatctaagcctggtcaggcatcagttcccctttttttgtgatttattttgtttttattttgttgttcattgtttaatttttccttttacaatgagaaggtcaccatcttgactcctaccttagccatttgttgaatcagactcatgacggctcctgggaagaagccagttcagatcataaaataaaacatatttattctttgtcatgggagtcattattttagaaactacaaactctccttgcttccatccttttttacatactcatgacacatgctcatcctgagtccttgaaaaggtatttttgaacatgtgtattaattataagcctctgaaaacctatggcccaaaccagaaatgatgttgattatataggtaaatgaaggatgctattgctgttctaattacctcattgtctcagtctcaaagtaggtcttcagctccctgtactttgggattttaatctaccaccacccataaatcaataaataattactttctttga

SEQ ID NO: 11 - RNA, 3975 nt, synthetic construct
  source 1..3975: mol_type = other RNA
cctttgccttcggacttctccggggccagcagccgcccgaccaggggcccggggccacgggctcagccgacgaccatgggctccgtgtccaaccagcagtttgcaggtggctgcgccaaggcggcagaagaggcgcccgaggaggcgccggaggacgcggcccgggcggcggacgagcctcagctgctgcacggtgcgggcatctgtaagtggttcaacgtgcgcatggggttcggcttcctgtccatgaccgcccgcgccggggtcgcgctcgaccccccagtggatgtctttgtgcaccagagtaagctgcacatggaagggttccggagcttgaaggagggtgaggcagtggagttcacctttaagaagtcagccaagggtctggaatccatccgtgtcaccggacctggtggagtattctgtattgggagtgagaggcggccaaaaggaaagagcatgcagaagcgcagatcaaaaggagacaggtgctacaactgtggaggtctagatcatcatgccaaggaatgcaagctgccaccccagcccaagaagtgccacttctgccagagcatcagccatatggtagcctcatgtccgctgaaggcccagcagggccctagtgcacagggaaagccaacctactttcgagaggaagaagaagaaatccacagccctaccctgctcccggaggcacagaattgagccacaatgggtgggggctattcttttgctatcaggaagttttgaggagcaggcagagtggagaaagtgggaatagggtgcattggggctagttggcactgccatgtatctcaggcttgggttcacaccatcaccctttcttccctctaggtggggggaaagggtgagtcaaaggaactccaaccatgctctgtccaaatgcaagtgagggttctgggggcaaccaggaggggggaatcaccctacaacctgcatactttgagtctccatccccagaatttccagcttttgaaagtggcctggatagggaagttgttttccttttaaagaaggatatataataattcccatgccagagtgaaatgattaagtataagaccagattcatggagccaagccactacattctgtggaaggagatctctcaggagtaagcattgtttttttttcacatcttgtatcctcatacccacttttgggatagggtgctggcagctgtcccaagcaatgggtaatgatgatggcaaaaagggtgtttgggggaacagctgcagacctgctgctctatgctcacccccgccccattctgggccaatgtgattttatttatttgctcccttggatactgcaccttgggtcccactttctccaggatgccaactgcactagctgtgtgcgaatgacgtatcttgtgcattttaactttttttccttaatataaatattctggttttgtatttttgtatattttaatctaaggccctcatttcctgcactgtgttctcaggtacatgagcaatctcagggatagccagcagcagctccaggtctgcgcagcaggaattactttttgttgtttttgccaccgtggagagcaactatttggagtgcacagcctattgaactacctcatttttgccaataagagctggcttttctgccatagtgtcctcttgaaaccccctctgccttgaaaatgttttatgggagactaggttttaactgggtggccccatgacttgattgccttctactggaagattgggaattagtctaaacaggaaatggtggtacacagaggctaggagaggctgggcccggtgaaaaggccagagagcaagccaagattaggtgagggttgtctaatcctatggcacaggacgtgctttacatctccagatctgttcttcaccagattaggttaggcctaccatgtgccacagggtgtgtgtgtgtttgtaaaactagagttgctaaggataagtttaaagaccaatacccctgtacttaatcctgtgctgtcgagggatggatatatgaagtaaggtgagatccttaacctttcaaaattttcgggttccagggagacacacaagcgagggttttgtggtgcctggagcctgtgtcctgccctgctacagtagtgattaatagtgtcatggtagctaaaggagaaaaagggggtttcgtttacacgctgtgagatcaccgcaaacctaccttactgtgttgaaacgggacaaatgcaatagaacgcattgggtggtgtgtgtctgatcctgggttcttgtctcccctaaatgctgccccccaagttactgtatttgtctgggctttgtaggacttcactacgttgattgctaggtggcctagtttgtgtaaatataatgtattggtctttctccgtgttctttgggggttttgtttacaaacttctttttgtattgagagaaaaatagccaaagcatctttgacagaaggttctgcaccaggcaaaaagatctgaaacattagtttggggggccctcttcttaaagtggggatcttgaaccatcctttcttttgtattccccttcccctattacctattagaccagatcttctgtcctaaaaacttgtcttctaccctgccctcttttctgttcacccccaaaagaaaacttacacacccacacacatacacatttcatgcttggagtgtctccacaactcttaaatgatgtatgcaaaaatactgaagctaggaaaaccctccatcccttgttcccaacctcctaagtcaagaccattaccatttctttctttcttttttttttttttttaaaatggagtctcactgtgtcacccaggctggagtgcagtggcatgatcggctcactgcagcctctgcctcttgggttcaagtgattctcctgcctcagcctcctgagtagctgggatttcaggcacccgccacactcagctaatttttgtatttttagtagagacggggtttcaccatgttgtccaggctggtctggaactcctgacctcaggtgatctgcccaccttggcttcccaaagtgctgggattacaggcatgagccaccatgctgggccaaccatttcttggtgtattcatgccaaacacttaagacactgctgtagcccaggcgcggtggctcacacctgtaatcccagcactttggaaggctgaggcgggcggatcacaaggtcacgagttcaaaactatcctggccaacacagtgaaaccccgtctctactaaaatacaaaaaaattagccgggtgtggtggtgcatgcctttagtcctagctattcaggaggctgaggcaggggaatcgcttgaacccgagaggcagaggttgcagtgagctgagatcgcaccactgcactccagcctggttacagagcaagactctgtctcaaacaaaacaaaacaaaacaaaaacacactactgtattttggatggatcaaacctccttaattttaatttctaatcctaaagtaaagagatgcaattgggggccttccatgtagaaagtggggtcaggaggccaagaaagggaatatgaatgtatatccaagtcactcaggaacttttatgcaggtgctagaaactttatgtcaaagtggccacaagattgtttaataggagacgaacgaatgtaactccatgtttactgctaaaaaccaaagctttgtgtaaaatcttgaatttatggggcgggagggtaggaaagcctgtacctgtctgtttttttcctgatccttttccctcattcctgaactgcaggagactgagcccctttgggctttggtgaccccatcactggggtgtgtttatttgatggttgattttgctgtactgggtacttcctttcccattttctaatcattttttaacacaagctgactcttcccttcccttctcctttccctgggaaaatacaatgaataaataaagacttattggtacgcaaactgtca

SEQ ID NO: 12 - RNA, 2809 nt, synthetic construct
  source 1..2809: mol_type = other RNA
actgtgtactgagactggatgcatccttgcaataaaaaagaggttgatcacgacaaatgtgaaccccgccgttataaaaacagccatcatggctgtaaatgccaaaaagcagtcagtcttgtaacttgaaaaaaaaaaaaaaggaattgtagattgtgcgcatggactcggagtgggggcggtggacagtaagtcatgatgttttggtggtaccacctggttgaatttcttcatctgaataagaagctcctgtgatgttctggggaggccttggaaggctagcgcatccctcatagaaagtgaatgggagctacggacaccgtaccccgggctcagagaagagcctgctggacctggaccttgctgagggccctggccccacctgctgccagggcctgtttctccctgcaggaagcccaccgccccgggctcacccccaagcttgtgagaggctgctgcatttcccccaccctgacaggtcacctagaccccaggccacgtatgtgaacggcagcctcccaaccacacaacacatcaaacaggagtccttgcccgactaccaagccatggcagaggcccgcacatccctgtctgcccactgtcggggcccgctggccactggcctgcacccagacctggacctcccgggccgaagcctcgccacccctgcgccttcctgctaccttctgggcagcgaacccagctctggcctgggcctccagcccgagacccacctccccgagggcagcctgaagcggtgctgcgtcttgggcctaccccccacctccccagcctcctcctcaccctgtgcctcctccgacgtcacctccatcatccgctcctcccagacgtctctggtcacctgtgtaaatggactccggagcccccctctgacgggagatctggggggcccttccaagcgggcccggcctggccctgcatcgacggacagccatgagggcagcttgcaacttgaagcctgccggaaggcgagcttcctgaagcaggaacccgcggatgagttttcagagctctttgggcctcaccagcagggcctgccgcccccctatcccctgtctcagttgccgcctggcccaagccttggaggcctggggctgggcctggcaggcagggtggtggccgggcggcaggcgtgccgctgggtggactgctgtgcagcctatgagcagcaggaggagctggtgcggcacatcgagaagagccacatcgaccagcgcaagggcgaggacttcacctgcttctgggctggctgcgtgcgccgctacaagcccttcaacgcccgctacaagctgctcatccacatgcgagtgcactcgggcgagaagcccaacaagtgcatgtttgaaggctgcagcaaggccttctcacggctggagaacctcaagatccacctgaggagccacacgggcgagaagccgtacctgtgccagcacccgggttgccagaaggccttcagcaactccagcgaccgcgccaagcaccagcgcacccacctagacacgaagccgtacgcctgtcagatccctggctgctccaagcgctacacagaccccagctccctccgcaagcacgtcaaggcccattcagccaaagagcagcaggtgcgtaagaagctgcatgcgggccctgacaccgaggccgacgtcctgaccgagtgtctggtcctgcagcagctccacacgtccacacagctggctgccagcgacggcaagggtggctgtggcctgggccaggagctgctcccaggtgtgtatcctggctccatcaccccccataacggacttgcatcgggcctcctgcccccagcgcacgacgtaccttccaggcaccacccgctggatgccaccaccagttcccaccaccatctgtcccctctgcccatggctgagagcacccgggatgggttggggcccggcctcctctcaccaatagtcagccccctgaaggggctggggccaccgccgctgcccccatcctctcagagccattctccggggggccagcccttccccacactccccagcaagccgtcctacccacccttccagagccctccacccccgcctctgcccagcccacaaggttaccagggcagtttccactccatccagagttgcttcccctatggcgactgctaccggatggctgaaccagcagccggtggggacggactggtcggggagacccacggtttcaaccccctgcggcccaatggctaccacagcctcagcacgcccttgcctgccacaggctatgaggccctggctgaggcctcatgccccacagcgctgccacagcagccatctgaagatgtggtgtccagcggccccgaggactgtggcttcttccccaatggagcctttgaccactgcctgggccacatcccctccatctacacagacacctgaaggagcccccacatgcgcctgcccatccagcactgcagatgccacctcgcccacctgctgtcgctcccaccctccgtgcacctagcaggagtgccaggccacagccggaacagccaggccatgacccaggggagccagcgctgccaccccacccagcgctgccagggagccgccatccgagcttgagctgggcgcacagaggtgcccgccaggatctgtggccctgtaacattccctcgatcttgtcttcccgttcctccccgcagtggttttgaaatcacagacctcgtgtatataaaatatgcagaacttgttttccgttcccctgccagttttatatttttggttttacaagaaaaaacattaaaaactggaaagga

SEQ ID NO: 13 - protein, 305 aa, Homo sapiens
MSVDPACPQSLPCFEASDCKESSPMPVICGPEENYPSLQMSSAEMPHTETVSPLPSSMDLLIQDSPDSSTSPKGKQPTSAEKSVAKKEDKVPVKKQKTRTVFSSTQLCVLNDRFQRQKYLSLQQMQELSNILNLSYKQVKTWFQNQRMKSKRWQKNNWPKNSNGVTQKASAPTYPSLYSSYHQGCLVNPTGNLPMWSNQTWNNSTWSNQTQNIQSWSNHSWNTQTWCTQSWNNQAWNSPFYNCGEESLQSCMQFQPNSPASDLEAALEAAGEGLNVIQQTTRYFSTPQTMDLFLNYSMNMQPEDV

SEQ ID NO: 14 - RNA, 2048 nt, synthetic construct
  source 1..2048: mol_type = other RNA
ataaatctagagactccaggattttaacgttctgctggactgagctggttgcctcatgttattatgcaggcaactcactttatcccaatttcttgatacttttccttctggaggtcctatttctctaacatcttccagaaaagtcttaaagctgccttaaccttttttccagtccacctcttaaattttttcctcctcttcctctatactaacatgagtgtggatccagcttgtccccaaagcttgccttgctttgaagcatccgactgtaaagaatcttcacctatgcctgtgatttgtgggcctgaagaaaactatccatccttgcaaatgtcttctgctgagatgcctcacacggagactgtctctcctcttccttcctccatggatctgcttattcaggacagccctgattcttccaccagtcccaaaggcaaacaacccacttctgcagagaagagtgtcgcaaaaaaggaagacaaggtcccggtcaagaaacagaagaccagaactgtgttctcttccacccagctgtgtgtactcaatgatagatttcagagacagaaatacctcagcctccagcagatgcaagaactctccaacatcctgaacctcagctacaaacaggtgaagacctggttccagaaccagagaatgaaatctaagaggtggcagaaaaacaactggccgaagaatagcaatggtgtgacgcagaaggcctcagcacctacctaccccagcctttactcttcctaccaccagggatgcctggtgaacccgactgggaaccttccaatgtggagcaaccagacctggaacaattcaacctggagcaaccagacccagaacatccagtcctggagcaaccactcctggaacactcagacctggtgcacccaatcctggaacaatcaggcctggaacagtcccttctataactgtggagaggaatctctgcagtcctgcatgcagttccagccaaattctcctgccagtgacttggaggctgccttggaagctgctggggaaggccttaatgtaatacagcagaccactaggtattttagtactccacaaaccatggatttattcctaaactactccatgaacatgcaacctgaagacgtgtgaagatgagtgaaactgatattactcaatttcagtctggacactggctgaatccttcctctcccctcctcccatccctcataggatttttcttgtttggaaaccacgtgttctggtttccatgatgcccatccagtcaatctcatggagggtggagtatggttggagcctaatcagcgaggtttctttttttttttttttcctattggatcttcctggagaaaatactttttttttttttttttttgaaacggagtcttgctctgtcgcccaggctggagtgcagtggcgcggtcttggctcactgcaagctccgtctcccgggttcacgccattctcctgcctcagcctcccgagcagctgggactacaggcgcccgccacctcgcccggctaatattttgtatttttagtagagacggggtttcactgtgttagccaggatggtctcgatctcctgaccttgtgatccacccgcctcggcctccctaacagctgggatttacaggcgtgagccaccgcgccctgcctagaaaagacattttaataaccttggctgccgtctctggctatagataagtagatctaatactagtttggatatctttagggtttagaatctaacctcaagaataagaaatacaagtacaaattggtgatgaagatgtattcgtattgtttgggattgggaggctttgcttattttttaaaaactattgaggtaaagggttaagctgtaacatacttaattgatttcttaccgtttttggctctgttttgctatatcccctaatttgttggttgtgctaatctttgtagaaagaggtctcgtatttgctgcatcgtaatgacatgagtactgctttagttggtttaagttcaaatgaatgaaacaactatttttcctttagttgattttac